European Patent Specification EP 3 132 025 B1, published August 30, 2023. Title: METHODS AND COMPOSITIONS FOR MODIFYING GENOMIC DNA. Applicant: LI, LINHONG PESHWA, MADHUSUDAN. Application UNKNOWN. The sequence listing filed with the application follows.

SEQUENCE LISTING (43 sequences)

SEQ ID NO: 1 - DNA, 11 bp, Artificial Sequence
  Synthetic Primer
  misc_feature (4)..(8): n is a, c, g, or t
gacnnnnngtc

SEQ ID NO: 2 - DNA, 13 bp, Artificial Sequence
  Synthetic Primer
  misc_feature (1)..(1): n is a, c, g, or t
  misc_feature (4)..(7): n is a, c, g, or t
  misc_feature (11)..(11): C or T
  misc_feature (13)..(13): n is a, c, g, or t
nacnnnngtaycn

SEQ ID NO: 3 - DNA, 12 bp, Artificial Sequence
  Synthetic Primer
  misc_feature (4)..(9): n is a, c, g, or t
cgannnnnntgc

SEQ ID NO: 4 - DNA, 11 bp, Artificial Sequence
  Synthetic Primer
  misc_feature (4)..(8): n is a, c, g, or t
gccnnnnnggc

SEQ ID NO: 5 - DNA, 10 bp, Artificial Sequence
  Synthetic Primer
  misc_feature (4)..(7): n is a, c, g, or t
gatnnnnatc

SEQ ID NO: 6 - DNA, 11 bp, Artificial Sequence
  Synthetic Primer
  misc_feature (3)..(9): n is a, c, g, or t
ccnnnnnnngg

SEQ ID NO: 7 - DNA, 11 bp, Artificial Sequence
  Synthetic Primer
  misc_feature (4)..(8): n is a, c, g, or t
gcannnnntgc

SEQ ID NO: 8 - DNA, 12 bp, Artificial Sequence
  Synthetic Primer
  misc_feature (4)..(9): n is a, c, g, or t
ccannnnnntgg

SEQ ID NO: 9 - DNA, 12 bp, Artificial Sequence
  Synthetic Primer
  misc_feature (4)..(9): n is a, c, g, or t
gacnnnnnngtc

SEQ ID NO: 10 - DNA, 11 bp, Artificial Sequence
  Synthetic Primer
  misc_feature (4)..(8): n is a, c, g, or t
cctnnnnnagg

SEQ ID NO: 11 - DNA, 10 bp, Artificial Sequence
  Synthetic Primer
  misc_feature (6)..(10): n is a, c, g, or t
gagtcnnnnn

SEQ ID NO: 12 - DNA, 10 bp, Artificial Sequence
  Synthetic Primer
  misc_feature (4)..(7): n is a, c, g, or t
  misc_feature (8)..(8): R = A or G
caynnnnrtg

SEQ ID NO: 13 - DNA, 11 bp, Artificial Sequence
  Synthetic Primer
  misc_feature (3)..(9): n is a, c, g, or t
gcnnnnnnngc

SEQ ID NO: 14 - DNA, 11 bp, Artificial Sequence
  Synthetic Primer
  misc_feature (4)..(8): n is a, c, g, or t
ccannnnntgg

SEQ ID NO: 15 - DNA, 10 bp, Artificial Sequence
  Synthetic Primer
  misc_feature (4)..(7): n is a, c, g, or t
gacnnnngtc

SEQ ID NO: 16 - DNA, 13 bp, Artificial Sequence
  Synthetic Primer
  misc_feature (5)..(9): n is a, c, g, or t
ggccnnnnnggcc

SEQ ID NO: 17 - DNA, 15 bp, Artificial Sequence
  Synthetic Primer
  misc_feature (4)..(12): n is a, c, g, or t
ccannnnnnnnntgg

SEQ ID NO: 18 - DNA, 10 bp, Artificial Sequence
  Synthetic Primer
  misc_feature (4)..(7): n is a, c, g, or t
gaannnnttc

SEQ ID NO: 19 - protein, 147 aa, Homo sapiens
MVHLTPEEKSAVTALWGKVNVDEVGGEALGRLLVVYPWTQRFFESFGDLSTPDAVMGNPKVKAHGKKVLGAFSDGLAHLDNLKGTFATLSELHCDKLHVDPENFRLLGNVLVCVLAHHFGKEFTPPVQAAYQKVVAGVANALAHKYH

SEQ ID NO: 20 - protein, 570 aa, Homo sapiens
MGNWAVNEGLSIFVILVWLGLNVFLFVWYYRVYDIPPKFFYTRKLLGSALALARAPAACLNFNCMLILLPVCRNLLSFLRGSSACCSTRVRRQLDRNLTFHKMVAWMIALHSAIHTIAHLFNVEWCVNARVNNSDPYSVALSELGDRQNESYLNFARKRIKNPEGGLYLAVTLLAGITGVVITLCLILIITSSTKTIRRSYFEVFWYTHHLFVIFFIGLAIHGAERIVRGQTAESLAVHNITVCEQKISEWGKIKECPIPQFAGNPPMTWKWIVGPMFLYLCERLVRFWRSQQKVVITKVVTHPFKTIELQMKKKGFKMEVGQYIFVKCPKVSKLEWHPFTLTSAPEEDFFSIHIRIVGDWTEGLFNACGCDKQEFQDAWKLPKIAVDGPFGTASEDVFSYEVVMLVGAGIGVTPFASILKSVWYKYCNNATNLKLKKIYFYWLCRDTHAFEWFADLLQLLESQMQERNNAGFLSYNIYLTGWDESQANHFAVHHDEEKDVITGLKQKTLYGRPNWDNEFKTIASQHPNTRIGVFLCGPEALAETLSKQSISNSESGPRGVHFIFNKENF

SEQ ID NO: 21 - DNA, 23 bp, Homo sapiens
ggggccactagggacaggattgg

SEQ ID NO: 22 - DNA, 20 bp, Artificial Sequence
  Synthetic Primer
ttcgggtcacctctcactcc

SEQ ID NO: 23 - DNA, 20 bp, Artificial Sequence
  Synthetic Primer
ggctccatcgtaagcaaacc

SEQ ID NO: 24 - DNA, 103 bp, Artificial Sequence
  Synthetic Primer
tacttttatctgtcccctccaccccacagtggggccactagggacagaagcttgattggtgacagaaaagccccatccttaggcctcctccttcctagtctcc

SEQ ID NO: 25 - DNA, 70 bp, Artificial Sequence
  Synthetic Primer
cctccaccccacagtggggccactagggacagaagcttgattggtgacagaaaagccccatccttaggcc

SEQ ID NO: 26 - DNA, 50 bp, Artificial Sequence
  Synthetic Primer
acagtggggccactagggacagaagcttgattggtgacagaaaagcccca

SEQ ID NO: 27 - DNA, 26 bp, Artificial Sequence
  Synthetic Primer
ctagggacagaagcttgattggtgac

SEQ ID NO: 28 - DNA, 23 bp, Artificial Sequence
  Synthetic Primer
agtctgccgttactgccctgtgg

SEQ ID NO: 29 - DNA, 146 bp, Artificial Sequence
  Synthetic Primer
tgacacaactgtgttcactagcaacctcaaacagacaccatggtgcatctgactcctgaagcttggagaagtctgccgttactgccctgtggggcaaggtgaacgtggatgaagttggtggtgaggccctgggcaggttggtatca

SEQ ID NO: 30 - DNA, 40 bp, Artificial Sequence
  Synthetic Primer
ttaatacgactcactataggagtctgccgttactgccctg

SEQ ID NO: 31 - DNA, 20 bp, Artificial Sequence
  Synthetic Primer
aaaagcaccgactcggtgcc

SEQ ID NO: 32 - DNA, 23 bp, Artificial Sequence
  Synthetic Primer
  misc_feature (21)..(21): n is a, c, g, or t
tttcctattactaaatgatcngg

SEQ ID NO: 33 - DNA, 23 bp, Artificial Sequence
  Synthetic Primer
  misc_feature (21)..(21): n is a, c, g, or t
cacccagatgaattgtacgtngg

SEQ ID NO: 34 - DNA, 23 bp, Artificial Sequence
  Synthetic Primer
  misc_feature (21)..(21): n is a, c, g, or t
tgcccacgtacaattcatctngg

SEQ ID NO: 35 - DNA, 23 bp, Artificial Sequence
  Synthetic Primer
  misc_feature (21)..(21): n is a, c, g, or t
agtccagatcatttagtaatngg

SEQ ID NO: 36 - DNA, 51 bp, Artificial Sequence
  Synthetic Primer
acatttttcacccagatgaattgtacgtgggcagaccgcagagagtttggc

SEQ ID NO: 37 - DNA, 99 bp, Artificial Sequence
  Synthetic Primer
ctattactaaatgatctggacttacatttttcacccagacgaattgtacgtgggcagaccgcagagagtttggctgtgcataatataacagtttgtgaa

SEQ ID NO: 38 - DNA, 146 bp, Artificial Sequence
  Synthetic Primer
tcttttaataaaacaatttaatttcctattactaaatgatctggacttacatttttcacccagatgaattgtacgtgggcagaccgcagagagtttggctgtgcataatataacagtttgtgaacaaaaaatctcagaatggggaa

SEQ ID NO: 39 - DNA, 196 bp, Artificial Sequence
  Synthetic Primer
cagagcacttaaaatatatgcagaatcttttaataaaacaatttaatttcctattactaaatgatctggacttacatttttcacccagatgaattgtacgtgggcagaccgcagagagtttggctgtgcataatataacagtttgtgaacaaaaaatctcagaatggggaaaaataaaggaatgcccaatccctca

SEQ ID NO: 40 - DNA, 42 bp, Artificial Sequence
  Synthetic Primer
atggtgcatctgactcctgtagtggagaagtctgccgttact

SEQ ID NO: 41 - DNA, 78 bp, Artificial Sequence
  Synthetic Primer
atggtgcatctgactcctgtggagaagtctgccgttacttaccacgtagactgaggacacctcttcagacggcaatga

SEQ ID NO: 42 - DNA, 39 bp, Artificial Sequence
  Synthetic Primer
atggtgcatctgactcctgaggagaagtctgccgttact

SEQ ID NO: 43 - DNA, 78 bp, Artificial Sequence; identical to SEQ ID NO: 41
  Synthetic Primer